European Patent Application EP 4 467 157 A1, published November 27, 2024. Title: PHARMACEUTICAL COMPOSITION FOR TREATING AT LEAST ONE DISORDER SELECTED FROM INFLAMMATORY BOWEL DISEASE AND INTESTINAL TUMOR. Applicant: TOKYO UNIVERSITY OF SCIENCE FOUNDATION. The sequence listing filed with the application follows.

SEQUENCE LISTING (112 sequences)

SEQ ID NO: 1 - DNA, 20 bp, synthetic construct
  misc_feature 1..20: note = synthesized primer sequence
  source 1..20: mol_type = other DNA
ttcaccaccatggagaaggc

SEQ ID NO: 2 - DNA, 20 bp, synthetic construct
  misc_feature 1..20: note = synthesized primer sequence
  source 1..20: mol_type = other DNA
ggcatggactgtggtcatga

SEQ ID NO: 3 - DNA, 21 bp, synthetic construct
  misc_feature 1..21: note = synthesized primer sequence
  source 1..21: mol_type = other DNA
tttaactcccttggcgcaaaa

SEQ ID NO: 4 - DNA, 20 bp, synthetic construct
  misc_feature 1..20: note = synthesized primer sequence
  source 1..20: mol_type = other DNA
ctttccctccgcattgacac

SEQ ID NO: 5 - DNA, 21 bp, synthetic construct
  misc_feature 1..21: note = synthesized primer sequence
  source 1..21: mol_type = other DNA
tgctactgttgatgttgggac

SEQ ID NO: 6 - DNA, 21 bp, synthetic construct
  misc_feature 1..21: note = synthesized primer sequence
  source 1..21: mol_type = other DNA
aatgccctggttttggttgaa

SEQ ID NO: 7 - DNA, 20 bp, synthetic construct
  misc_feature 1..20: note = synthesized primer sequence
  source 1..20: mol_type = other DNA
gcctccctctcatcagttct

SEQ ID NO: 8 - DNA, 20 bp, synthetic construct
  misc_feature 1..20: note = synthesized primer sequence
  source 1..20: mol_type = other DNA
cacttggtggtttgctacga

SEQ ID NO: 9 - DNA, 21 bp, synthetic construct
  misc_feature 1..21: note = synthesized primer sequence
  source 1..21: mol_type = other DNA
ggtcccctgtgagcccgcaac

SEQ ID NO: 10 - DNA, 27 bp, synthetic construct
  misc_feature 1..27: note = synthesized primer sequence
  source 1..27: mol_type = other DNA
tgactgtgcgtgagggatccactgact

SEQ ID NO: 11 - DNA, 23 bp, synthetic construct
  misc_feature 1..23: note = synthesized primer sequence
  source 1..23: mol_type = other DNA
gaggataccactcccaacagacc

SEQ ID NO: 12 - DNA, 24 bp, synthetic construct
  misc_feature 1..24: note = synthesized primer sequence
  source 1..24: mol_type = other DNA
aagtgcatcatcgttgttcataca

SEQ ID NO: 13 - DNA, 19 bp, synthetic construct
  misc_feature 1..19: note = synthesized primer sequence
  source 1..19: mol_type = other DNA
tccagggcagagagggagt

SEQ ID NO: 14 - DNA, 22 bp, synthetic construct
  misc_feature 1..22: note = synthesized primer sequence
  source 1..22: mol_type = other DNA
ggaactttggccatcttgattt

SEQ ID NO: 15 - DNA, 25 bp, synthetic construct
  misc_feature 1..25: note = synthesized primer sequence
  source 1..25: mol_type = other DNA
caaccaacaagtgatattctccatg

SEQ ID NO: 16 - DNA, 21 bp, synthetic construct
  misc_feature 1..21: note = synthesized primer sequence
  source 1..21: mol_type = other DNA
gatccacactctccagctgca

SEQ ID NO: 17 - DNA, 21 bp, synthetic construct
  misc_feature 1..21: note = synthesized primer sequence
  source 1..21: mol_type = other DNA
aatgccctggttttggttgaa

SEQ ID NO: 18 - DNA, 21 bp, synthetic construct
  misc_feature 1..21: note = synthesized primer sequence
  source 1..21: mol_type = other DNA
aatgccctggttttggttgaa

SEQ ID NO: 19 - DNA, 21 bp, synthetic construct
  misc_feature 1..21: note = synthesized primer sequence
  source 1..21: mol_type = other DNA
ggccttggaagcatgtagagg

SEQ ID NO: 20 - DNA, 23 bp, synthetic construct
  misc_feature 1..23: note = synthesized primer sequence
  source 1..23: mol_type = other DNA
ggagaactcgttagagacgactt

SEQ ID NO: 21 - DNA, 20 bp, synthetic construct
  misc_feature 1..20: note = synthesized primer sequence
  source 1..20: mol_type = other DNA
agaagctgggagctatgcag

SEQ ID NO: 22 - DNA, 20 bp, synthetic construct
  misc_feature 1..20: note = synthesized primer sequence
  source 1..20: mol_type = other DNA
tactggtggctacgatgcag

SEQ ID NO: 23 - DNA, 22 bp, synthetic construct
  misc_feature 1..22: note = synthesized primer sequence
  source 1..22: mol_type = other DNA
tgacgtcactggagttgtacgg

SEQ ID NO: 24 - DNA, 21 bp, synthetic construct
  misc_feature 1..21: note = synthesized primer sequence
  source 1..21: mol_type = other DNA
ggttcatgtcatggatggtgc

SEQ ID NO: 25 - DNA, 20 bp, synthetic construct
  misc_feature 1..20: note = synthesized primer sequence
  source 1..20: mol_type = other DNA
ggtgtctgggaagctgagag

SEQ ID NO: 26 - DNA, 20 bp, synthetic construct
  misc_feature 1..20: note = synthesized primer sequence
  source 1..20: mol_type = other DNA
ccacatccacaaacatcctg

SEQ ID NO: 27 - DNA, 20 bp, synthetic construct
  misc_feature 1..20: note = synthesized primer sequence
  source 1..20: mol_type = other DNA
gccgctaagagccacagcaa

SEQ ID NO: 28 - DNA, 22 bp, synthetic construct
  misc_feature 1..22: note = synthesized primer sequence
  source 1..22: mol_type = other DNA
gccctccttttaacacatcaga

SEQ ID NO: 29 - DNA, 21 bp, synthetic construct
  misc_feature 1..21: note = synthesized primer sequence
  source 1..21: mol_type = other DNA
ttcctctgaccttgagtgtgg

SEQ ID NO: 30 - DNA, 22 bp, synthetic construct
  misc_feature 1..22: note = synthesized primer sequence
  source 1..22: mol_type = other DNA
ctcttgccctttcctgctcttt

SEQ ID NO: 31 - DNA, 20 bp, synthetic construct
  misc_feature 1..20: note = synthesized primer sequence
  source 1..20: mol_type = other DNA
gtcctgggaatctccttggc

SEQ ID NO: 32 - DNA, 20 bp, synthetic construct
  misc_feature 1..20: note = synthesized primer sequence
  source 1..20: mol_type = other DNA
tctgtgccgtgacgatgttg

SEQ ID NO: 33 - DNA, 20 bp, synthetic construct
  misc_feature 1..20: note = synthesized primer sequence
  source 1..20: mol_type = other DNA
agagtttgatcmtggctcag

SEQ ID NO: 34 - DNA, 15 bp, synthetic construct
  misc_feature 1..15: note = synthesized primer sequence
  source 1..15: mol_type = other DNA
ctgctgcctyccgta

SEQ ID NO: 35 - DNA, 23 bp, synthetic construct
  misc_feature 1..23: note = synthesized primer sequence
  source 1..23: mol_type = other DNA
atgtgtagcggtaaaatgcgtaa

SEQ ID NO: 36 - DNA, 21 bp, synthetic construct
  misc_feature 1..21: note = synthesized primer sequence
  source 1..21: mol_type = other DNA
cmtacttgcgtaggtactact

SEQ ID NO: 37 - DNA, 21 bp, synthetic construct
  misc_feature 1..21: note = synthesized primer sequence
  source 1..21: mol_type = other DNA
tgaaactyaaaggaattgacg

SEQ ID NO: 38 - DNA, 17 bp, synthetic construct
  misc_feature 1..17: note = synthesized primer sequence
  source 1..17: mol_type = other DNA
accatgcaccacctgtc

SEQ ID NO: 39 - DNA, 22 bp, synthetic construct
  misc_feature 1..22: note = synthesized primer sequence
  source 1..22: mol_type = other DNA
taggcttgacattgatagaatc

SEQ ID NO: 40 - DNA, 21 bp, synthetic construct
  misc_feature 1..21: note = synthesized primer sequence
  source 1..21: mol_type = other DNA
cttacgaaggcagtctcctta

SEQ ID NO: 41 - DNA, 16 bp, synthetic construct
  misc_feature 1..16: note = synthesized primer sequence
  source 1..16: mol_type = other DNA
tacggccgcaaggcta

SEQ ID NO: 42 - DNA, 19 bp, synthetic construct
  misc_feature 1..19: note = synthesized primer sequence
  source 1..19: mol_type = other DNA
tcrtccccaccttcctccg

SEQ ID NO: 43 - DNA, 19 bp, synthetic construct
  misc_feature 1..19: note = synthesized primer sequence
  modified_base 2: mod_base = i
  source 1..19: mol_type = other DNA
cnagtgtagaggtgaaatt

SEQ ID NO: 44 - DNA, 21 bp, synthetic construct
  misc_feature 1..21: note = synthesized primer sequence
  source 1..21: mol_type = other DNA
ccccgtcaattcctttgagtt

SEQ ID NO: 45 - DNA, 19 bp, synthetic construct
  misc_feature 1..19: note = synthesized primer sequence
  source 1..19: mol_type = other DNA
caccaaggcgacgatcagt

SEQ ID NO: 46 - DNA, 19 bp, synthetic construct
  misc_feature 1..19: note = synthesized primer sequence
  source 1..19: mol_type = other DNA
gagtttgggccgtgtctca

SEQ ID NO: 47 - DNA, 19 bp, synthetic construct
  misc_feature 1..19: note = synthesized primer sequence
  source 1..19: mol_type = other DNA
tcgtcagctcgtgtygtga

SEQ ID NO: 48 - DNA, 16 bp, synthetic construct
  misc_feature 1..16: note = synthesized primer sequence
  source 1..16: mol_type = other DNA
cgtaagggccatgatg

SEQ ID NO: 49 - DNA, 21 bp, synthetic construct
  misc_feature 1..21: note = synthesized primer sequence
  source 1..21: mol_type = other DNA
tggaaacagrtgctaataccg

SEQ ID NO: 50 - DNA, 20 bp, synthetic construct
  misc_feature 1..20: note = synthesized primer sequence
  source 1..20: mol_type = other DNA
gtccattgtggaagattccc

SEQ ID NO: 51 - DNA, 75 bp, Mus musculus
  source 1..75: mol_type = other DNA
gaggtgaagcttctcgagtctggaggtggcctggtgcagcctggaggatccctgaaactctcctgtgcagcctca

SEQ ID NO: 52 - DNA, 24 bp, Mus musculus
  source 1..24: mol_type = other DNA
ggattcgattttagtagatactgg

SEQ ID NO: 53 - DNA, 51 bp, Mus musculus
  source 1..51: mol_type = other DNA
atgagttgggtccggcaggctccagggaaagggctagaatggattggagaa

SEQ ID NO: 54 - DNA, 24 bp, Mus musculus
  source 1..24: mol_type = other DNA
attaatccagatagcagtacgata

SEQ ID NO: 55 - DNA, 114 bp, Mus musculus
  source 1..114: mol_type = other DNA
aactatacgccatctctaaaggataaattcatcatctccagagacaacgccaaaaatacgctgtacctgcaaatgagcaaagtgagatctgaggacacagccctttattactgt

SEQ ID NO: 56 - DNA, 51 bp, Mus musculus
  source 1..51: mol_type = other DNA
gcaagacctgatgggacgatttattactacggttgctggtacttcgatgtc

SEQ ID NO: 57 - DNA, 21 bp, Mus musculus
  source 1..21: mol_type = other DNA
tggggcgcagggaccacggtc

SEQ ID NO: 58 - DNA, 78 bp, Mus musculus
  source 1..78: mol_type = other DNA
gatgttgtgatgacccaaactccactctccctgcctgtcagtctgggagatcaagcctccatctcttgcagatctagt

SEQ ID NO: 59 - DNA, 33 bp, Mus musculus
  source 1..33: mol_type = other DNA
cagagtcttgcacacagtaatggaaacacctat

SEQ ID NO: 60 - DNA, 51 bp, Mus musculus
  source 1..51: mol_type = other DNA
ttacattggtacctgcagaagccaggccagtctccaaagctcctgatctac

SEQ ID NO: 61 - DNA, 108 bp, Mus musculus
  source 1..108: mol_type = other DNA
aaccgattttctggggtcccagacaggttcagtggcagtggatcagggacagatttcacactcaagatcagcagagtggaggctgaggatctgggagtttatttctgc

SEQ ID NO: 62 - DNA, 27 bp, Mus musculus
  source 1..27: mol_type = other DNA
tctcaaagtacacatgttccgtggacg

SEQ ID NO: 63 - DNA, 30 bp, Mus musculus
  source 1..30: mol_type = other DNA
ttcggtggaggcaccaagctggaaatcaaa

SEQ ID NO: 64 - protein, 25 aa, Mus musculus
EVKLLESGGGLVQPGGSLKLSCAAS

SEQ ID NO: 65 - protein, 8 aa, Mus musculus
GFDFSRYW

SEQ ID NO: 66 - protein, 17 aa, Mus musculus
MSWVRQAPGKGLEWIGE

SEQ ID NO: 67 - protein, 8 aa, Mus musculus
INPDSSTI

SEQ ID NO: 68 - protein, 38 aa, Mus musculus
NYTPSLKDKFIISRDNAKNTLYLQMSKVRSEDTALYYC

SEQ ID NO: 69 - protein, 17 aa, Mus musculus
ARPDGTIYYYGCWYFDV

SEQ ID NO: 70 - protein, 7 aa, Mus musculus
WGAGTTV

SEQ ID NO: 71 - protein, 26 aa, Mus musculus
DVVMTQTPLSLPVSLGDQASISCRSS

SEQ ID NO: 72 - protein, 11 aa, Mus musculus
QSLAHSNGNTY

SEQ ID NO: 73 - protein, 17 aa, Mus musculus
LHWYLQKPGQSPKLLIY

SEQ ID NO: 74 - protein, 36 aa, Mus musculus [sequence omitted]

SEQ ID NO: 75 - protein, 9 aa, Mus musculus
SQSTHVPWT

SEQ ID NO: 76 - protein, 10 aa, Mus musculus
FGGGTKLEIK

SEQ ID NO: 77 - DNA, 360 bp, Mus musculus
  source 1..360: mol_type = other DNA
gaggtgaagcttctcgagtctggaggtggcctggtgcagcctggaggatccctgaaactctcctgtgcagcctcaggattcgattttagtagatactggatgagttgggtccggcaggctccagggaaagggctagaatggattggagaaattaatccagatagcagtacgataaactatacgccatctctaaaggataaattcatcatctccagagacaacgccaaaaatacgctgtacctgcaaatgagcaaagtgagatctgaggacacagccctttattactgtgcaagacctgatgggacgatttattactacggttgctggtacttcgatgtctggggcgcagggaccacggtc

SEQ ID NO: 78 - DNA, 336 bp, Mus musculus
  source 1..336: mol_type = other DNA
gatgttgtgatgacccaaactccactctccctgcctgtcagtctgggagatcaagcctccatctcttgcagatctagtcagagtcttgcacacagtaatggaaacacctatttacattggtacctgcagaagccaggccagtctccaaagctcctgatctacaaaatttccaaccgattttctggggtcccagacaggttcagtggcagtggatcagggacagatttcacactcaagatcagcagagtggaggctgaggatctgggagtttatttctgctctcaaagtacacatgttccgtggacgttcggtggaggcaccaagctggaaatcaaa

SEQ ID NO: 79 - protein, 120 aa, Mus musculus
EVKLLESGGGLVQPGGSLKLSCAASGFDFSRYWMSWVRQAPGKGLEWIGEINPDSSTINYTPSLKDKFIISRDNAKNTLYLQMSKVRSEDTALYYCARPDGTIYYYGCWYFDVWGAGTTV

SEQ ID NO: 80 - protein, 112 aa, Mus musculus
DVVMTQTPLSLPVSLGDQASISCRSSQSLAHSNGNTYLHWYLQKPGQSPKLLIYKISNRFSGVPDRFSGSGSGTDFTLKISRVEAEDLGVYFCSQSTHVPWTFGGGTKLEIK

SEQ ID NO: 81 - DNA, 75 bp, Mus musculus
  source 1..75: mol_type = other DNA
gaggtccagctgcagcagtctggacctgagctggtaaagcctggggcttcagtgaagatgtcctgcaaggcttct

SEQ ID NO: 82 - DNA, 24 bp, Mus musculus
  source 1..24: mol_type = other DNA
ggatacacattcactagctatgtt

SEQ ID NO: 83 - DNA, 51 bp, Mus musculus
  source 1..51: mol_type = other DNA
atgcactgggtgaagcagaagcctgggcagggccttgagtggattggatat

SEQ ID NO: 84 - DNA, 24 bp, Mus musculus
  source 1..24: mol_type = other DNA
attaatccttacaatgatggtact

SEQ ID NO: 85 - DNA, 114 bp, Mus musculus
  source 1..114: mol_type = other DNA
aagtacaatgagaagttcaaaggcaaggccacactgacttcagacaaatcctccagcacagcctacatggagctcagcagcctgacctctgaggactatgcggtctattactgt

SEQ ID NO: 86 - DNA, 36 bp, Mus musculus
  source 1..36: mol_type = other DNA
gcaagatcctacaagaggtacgactggtacccaaga

SEQ ID NO: 87 - DNA, 21 bp, Mus musculus
  source 1..21: mol_type = other DNA
tggggcgcagggaccacggtc

SEQ ID NO: 88 - DNA, 78 bp, Mus musculus
  source 1..78: mol_type = other DNA
gacattgtgatgacccagtctcaaaaattcatgtccacatcagtaggagacagggtcagcgtcacctgcaaggccagt

SEQ ID NO: 89 - DNA, 18 bp, Mus musculus
  source 1..18: mol_type = other DNA
cagaatgtgggtactaat

SEQ ID NO: 90 - DNA, 51 bp, Mus musculus
  source 1..51: mol_type = other DNA
gtagcctggtatcaacagaaaccagggcaatctcctaaagcactgatttac

SEQ ID NO: 91 - skipped

SEQ ID NO: 92 - DNA, 108 bp, Mus musculus
  source 1..108: mol_type = other DNA
taccggtacagtggagtccctgatcgcttcacaggcagtggatctgggacagatttcactctcaccatcagcaatgtgcagtctgaagacttggcagagtatttctgt

SEQ ID NO: 93 - DNA, 27 bp, Mus musculus
  source 1..27: mol_type = other DNA
cagcaatataacagctatccgctcacg

SEQ ID NO: 94 - DNA, 30 bp, Mus musculus; identical to SEQ ID NO: 63
  source 1..30: mol_type = other DNA

SEQ ID NO: 95 - protein, 25 aa, Mus musculus
EVQLQQSGPELVKPGASVKMSCKAS

SEQ ID NO: 96 - protein, 8 aa, Mus musculus
GYTFTSYV

SEQ ID NO: 97 - protein, 17 aa, Mus musculus
MHWVKQKPGQGLEWIGY

SEQ ID NO: 98 - protein, 8 aa, Mus musculus
INPYNDGT

SEQ ID NO: 99 - protein, 38 aa, Mus musculus
KYNEKFKGKATLTSDKSSSTAYMELSSLTSEDYAVYYC

SEQ ID NO: 100 - protein, 12 aa, Mus musculus
ARSYKRYDWYPR

SEQ ID NO: 101 - protein, 7 aa, Mus musculus
WGAGTTV

SEQ ID NO: 102 - protein, 26 aa, Mus musculus
DIVMTQSQKFMSTSVGDRVSVTCKAS

SEQ ID NO: 103 - protein, 6 aa, Mus musculus
QNVGTN

SEQ ID NO: 104 - protein, 17 aa, Mus musculus
VAWYQQKPGQSPKALIY

SEQ ID NO: 105 - skipped

SEQ ID NO: 106 - protein, 36 aa, Mus musculus
YRYSGVPDRFTGSGSGTDFTLTISNVQSEDLAEYFC

SEQ ID NO: 107 - protein, 9 aa, Mus musculus
QQYNSYPLT

SEQ ID NO: 108 - protein, 10 aa, Mus musculus
FGGGTKLEIK

SEQ ID NO: 109 - DNA, 345 bp, Mus musculus
  source 1..345: mol_type = other DNA
gaggtccagctgcagcagtctggacctgagctggtaaagcctggggcttcagtgaagatgtcctgcaaggcttctggatacacattcactagctatgttatgcactgggtgaagcagaagcctgggcagggccttgagtggattggatatattaatccttacaatgatggtactaagtacaatgagaagttcaaaggcaaggccacactgacttcagacaaatcctccagcacagcctacatggagctcagcagcctgacctctgaggactatgcggtctattactgtgcaagatcctacaagaggtacgactggtacccaagatggggcgcagggaccacggtc

SEQ ID NO: 110 - DNA, 321 bp, Mus musculus
  source 1..321: mol_type = other DNA
gacattgtgatgacccagtctcaaaaattcatgtccacatcagtaggagacagggtcagcgtcacctgcaaggccagtcagaatgtgggtactaatgtagcctggtatcaacagaaaccagggcaatctcctaaagcactgatttactcggcatcctaccggtacagtggagtccctgatcgcttcacaggcagtggatctgggacagatttcactctcaccatcagcaatgtgcagtctgaagacttggcagagtatttctgtcagcaatataacagctatccgctcacgttcggtggaggcaccaagctggaaatcaaa

SEQ ID NO: 111 - protein, 115 aa, Mus musculus
EVQLQQSGPELVKPGASVKMSCKASGYTFTSYVMHWVKQKPGQGLEWIGYINPYNDGTKYNEKFKGKATLTSDKSSSTAYMELSSLTSEDYAVYYCARSYKRYDWYPRWGAGTTV

SEQ ID NO: 112 - protein, 107 aa, Mus musculus
DIVMTQSQKFMSTSVGDRVSVTCKASQNVGTNVAWYQQKPGQSPKALIYSASYRYSGVPDRFTGSGSGTDFTLTISNVQSEDLAEYFCQQYNSYPLTFGGGTKLEIK